European Patent Application EP 4 321 528 A1, published February 14, 2024. Title: Peptide for preventing or treating inflammatory diseases. Applicant: AJOU UNIVERSITY INDUSTRY-ACADEMIC COOPERATION FOUNDATION. The sequence listing filed with the application follows.

SEQUENCE LISTING (7 sequences)

SEQ ID NO: 1 - protein, 13 aa, Artificial Sequence
  P1
LICPEKYCNKVHT

SEQ ID NO: 2 - protein, 11 aa, Artificial Sequence
  P2
YCNKVHTCRNG

SEQ ID NO: 3 - protein, 11 aa, Artificial Sequence
  P4
HTCRNGENICF

SEQ ID NO: 4 - protein, 22 aa, Artificial Sequence
  E1
LICPEKYCNKVHTCRNGENICF

SEQ ID NO: 5 - protein, 25 aa, Artificial Sequence
  E2
LTCLICPEKYCNKVHTCRNGENICF

SEQ ID NO: 6 - protein, 21 aa, Artificial Sequence
  E3
TCPEAKPREIVECCSTDKCNH

SEQ ID NO: 7 - protein, 25 aa, Artificial Sequence
  E4
GCAATCPEAKPREIVECCSTDKCNH